European Patent Application EP 4 467 153 A1, published November 27, 2024. Title: CONSTRAINED PEPTIDE INHIBITORS OF LRRK2-FADD INTERACTIONS. Applicant: University of Georgia Research Foundation, Inc. The sequence listing filed with the application follows.

SEQUENCE LISTING (8 sequences)

SEQ ID NO: 1 - protein, 20 aa, synthetic construct
  source 1..20: note = alpha-helix forming peptide
  VARIANT 1: note = Optionally wherein the N-terminal lysine is conjugated to PEG3
KVADLVQEVQQARDLQNRSK

SEQ ID NO: 2 - protein, 20 aa, synthetic construct
  source 1..20: note = alpha-helix forming peptide variant
  VARIANT 2: note = X is (S)-2-(4-pentenyl)alanine
  VARIANT 6: note = X is (S)-2-(4-pentenyl)alanine
  VARIANT 1: note = Optionally wherein the N-terminal lysine is conjugated to 5(6)FAM-PEG3 or PEG3
KXADLXQEVQQARDLQNRSK

SEQ ID NO: 3 - protein, 20 aa, synthetic construct
  source 1..20: note = alpha-helix forming peptide variant
  VARIANT 6: note = X is (S)-2-(4-pentenyl)alanine
  VARIANT 10: note = X is (S)-2-(4-pentenyl)alanine
  VARIANT 1: note = Optionally wherein the N-terminal lysine is conjugated to 5(6)FAM-PEG3 or PEG3
KVADLXQEVXQARDLQNRSK

SEQ ID NO: 4 - protein, 20 aa, synthetic construct
  source 1..20: note = alpha-helix forming peptide variant
  VARIANT 9: note = X is (S)-2-(4-pentenyl)alanine
  VARIANT 13: note = X is (S)-2-(4-pentenyl)alanine
  VARIANT 1: note = Optionally wherein the N-terminal lysine is conjugated to 5(6)FAM-PEG3 or PEG3
KVADLVQEXQQAXDLQNRSK

SEQ ID NO: 5 - protein, 20 aa, synthetic construct
  source 1..20: note = alpha-helix forming peptide variant
  VARIANT 12: note = X is (S)-2-(4-pentenyl)alanine
  VARIANT 16: note = X is (S)-2-(4-pentenyl)alanine
  VARIANT 1: note = Optionally wherein the N-terminal lysine is conjugated to 5(6)FAM-PEG3 or PEG3
KVADLVQEVQQXRDLXNRSK

SEQ ID NO: 6 - protein, 20 aa, synthetic construct
  source 1..20: note = alpha-helix forming peptide variant
  VARIANT 13: note = X is (S)-2-(4-pentenyl)alanine
  VARIANT 17: note = X is (S)-2-(4-pentenyl)alanine
  VARIANT 1: note = Optionally wherein the N-terminal lysine is conjugated to 5(6)FAM-PEG3 or PEG3
KVADLVQEVQQAXDLQXRSK

SEQ ID NO: 7 - protein, 18 aa, synthetic construct
  source 1..18: note = FADD death-domain
VADLVQEVQQARDLQNRS

SEQ ID NO: 8 - protein, 18 aa, synthetic construct
  source 1..18: note = LRRK2 ARM domain
MVKKQCFKNDIHKLVLAA